European Patent Application EP 4 509 188 A2, published February 19, 2025. Title: MODIFIED ANTI-INFLAMMATORY PROTEINS AND METHOD OF USE. Applicant: James Cook University. Application EP PCT/AU2014/050240, filed September 18, 2014. The sequence listing filed with the application follows.

SEQUENCE LISTING (5 sequences)

SEQ ID NO: 1 - protein, 141 aa, synthetic construct
ACSCKPFGTLKEAFCQSDYVLLAKVLSVNSKYGESSRNEANDMSTTANGTWSYHVWHMRTWKGPVVDTSVLTTSYSECGVTGLLKNWDYFLTGKQGKDGEITITSCDFVMPSTDVTPEEHDLLMDLMGDPKKCEEKDDERD

SEQ ID NO: 2 - protein, 228 aa, synthetic construct
ACSCKPFGTLKEAFCQSDYVLLAKVLSVNSKYGESSRNEANDMSTTANGTWSYHVWHMRTWKGPVVDTSVLTTSYSECGVTGLLKNWDYFLTGKQGKDGEITITSCDFVMPSTDVTPEEHDLLMDLMGDPKKCEEKDDERDVKENENSVEENDEKDEEENGEKTVEENDEKTVEENDEKVEEENGEKTVEENDEKIVEENDEKDEEENGEKTVEENDEKTVEENDEQE

SEQ ID NO: 3 - DNA, 423 bp, synthetic construct
  source 1..423: mol_type = other DNA
gcatgctcttgcaaaccgttcggaacactgaaggaagctttctgccaatcagattacgtgcttctggcaaaagtgttgtcagtaaatagtaaatatggtgaatcgtcgagaaatgaagcaaatgatatgagcacgaccgctaacggaacatggagttaccatgtatggcacatgcggacttggaagggtcctgtcgttgatactagtgttctcaccacgtcatatagcgagtgtggtgtaactggtctcttgaaaaattgggattattttctaacaggcaagcaaggaaaagatggcgaaatcaccatcacaagctgcgactttgtaatgccatcaactgatgtcacaccagaagagcatgatcttttgatggacctcatgggggacccgaaaaaatgtgaagaaaaagatgatgagagggac

SEQ ID NO: 4 - protein, 228 aa, synthetic construct
ACSCKPFGTLKEAFCQSDYVLLAKVLSVNSKYGESSRNEANDMSTTAQGTWSYHVWHMRTWKGPVVDTSVLTTSYSECGVTGLLKNWDYFLTGKQGKDGEITITSCDFVMPSTDVTPEEHDLLMDLMGDPKKCEEKDDERDVKENENSVEENDEKDEEENGEKTVEENDEKTVEENDEKVEEENGEKTVEENDEKIVEENDEKDEEENGEKTVEENDEKTVEENDEQE

SEQ ID NO: 5 - protein, 141 aa, synthetic construct
ACSCKPFGTLKEAFCQSDYVLLAKVLSVNSKYGESSRNEANDMSTTAQGTWSYHVWHMRTWKGPVVDTSVLTTSYSECGVTGLLKNWDYFLTGKQGKDGEITITSCDFVMPSTDVTPEEHDLLMDLMGDPKKCEEKDDERD